European Patent Specification EP 3 802 621 B1, published July 30, 2025. Title: Composition and Application of Arginine-depleting Agents for Cancer, Obesity, Metabolic Disorders, and Related Complications and Comorbidities. Applicant: The Hong Kong Polytechnic University The Chinese University of Hong Kong. The sequence listing filed with the application follows.

SEQUENCE LISTING (106 sequences)

SEQ ID NO: 1 - DNA, 50 bp, Artificial Sequence
  ABD Primer 1, Synthesized in the Lab
ggagatggacatatgcatcatcaccatcaccatgatgaagccgtggatgc

SEQ ID NO: 2 - DNA, 50 bp, Artificial Sequence
  ABD Primer 2, Synthesized in the Lab
gctaagactttagcttcagctaaggaattcgcatccacggcttcatcatg

SEQ ID NO: 3 - DNA, 50 bp, Artificial Sequence
  ABD Primer 3, Synthesized in the Lab
ccttagctgaagctaaagtcttagctaacagagaacttgacaaatatgga

SEQ ID NO: 4 - DNA, 50 bp, Artificial Sequence
  ABD Primer 4, Synthesized in the Lab
taggttcttgtaatagtcacttactccatatttgtcaagttctctgttag

SEQ ID NO: 5 - DNA, 50 bp, Artificial Sequence
  ABD Primer 5, Synthesized in the Lab
ggagtaagtgactattacaagaacctaatcaacaatgccaaaactgttga

SEQ ID NO: 6 - DNA, 50 bp, Artificial Sequence
  ABD Primer 6, Synthesized in the Lab
aaatttcatctatcagtgcttttacaccttcaacagttttggcattgttg

SEQ ID NO: 7 - DNA, 50 bp, Artificial Sequence
  ABD Primer 7, Synthesized in the Lab
gtaaaagcactgatagatgaaattttagctgcattaccttcgggtagtaa

SEQ ID NO: 8 - DNA, 50 bp, Artificial Sequence
  ABD Primer 8, Synthesized in the Lab
tccgccgctaccattgttattattgttgttactacccgaaggtaatgcag

SEQ ID NO: 9 - DNA, 47 bp, Artificial Sequence
  ABD Primer 9, Synthesized in the Lab
gatcttaagcatatgcatcatcaccatcaccatgatgaagcggtgga

SEQ ID NO: 10 - DNA, 47 bp, Artificial Sequence
  ABD Primer 10, Synthesized in the Lab
gcttctttcgcttccgccaggctgttcgcatccaccgcttcatcatg

SEQ ID NO: 11 - DNA, 50 bp, Artificial Sequence
  ABD Primer 11, Synthesized in the Lab
gcggaagcgaaagaagcggcgaacgcggaactggatagctatggcgtgag

SEQ ID NO: 12 - DNA, 50 bp, Artificial Sequence
  ABD Primer 12, Synthesized in the Lab
ttatcaatcaggcgtttataaaaatcgctcacgccatagctatccagttc

SEQ ID NO: 13 - DNA, 50 bp, Artificial Sequence
  ABD Primer 13, Synthesized in the Lab
gatttttataaacgcctgattgataaagcgaaaaccgtggaaggcgtgga

SEQ ID NO: 14 - DNA, 51 bp, Artificial Sequence
  ABD Primer 14, Synthesized in the Lab
cggcagcgccgccagaatcgcatctttcagcgcttccacgccttccacggt

SEQ ID NO: 15 - DNA, 50 bp, Artificial Sequence
  ABD Primer 15, Synthesized in the Lab
ttctggcggcgctgccgtcgggtagtaacaacaataataacaatggtagc

SEQ ID NO: 16 - DNA, 39 bp, Artificial Sequence
  ABD Primer 16, Synthesized in the Lab
ggatccgccgctaccattgttattattgttgttactacc

SEQ ID NO: 17 - DNA, 50 bp, Artificial Sequence
  ABD Primer 17, Synthesized in the Lab
catatgttagctgatggatccagtaacaacaataataacaatggtagcgg

SEQ ID NO: 18 - DNA, 50 bp, Artificial Sequence
  ABD Primer 18, Synthesized in the Lab
aattcgcatccacggcttcatcaccgccgctaccattgttattattgttg

SEQ ID NO: 19 - DNA, 50 bp, Artificial Sequence
  ABD Primer 19, Synthesized in the Lab
gaagccgtggatgcgaattccttagctgaagctaaagtcttagctaacag

SEQ ID NO: 20 - DNA, 50 bp, Artificial Sequence
  ABD Primer 20, Synthesized in the Lab
cttactccatatttgtcaagttctctgttagctaagactttagcttcagc

SEQ ID NO: 21 - DNA, 50 bp, Artificial Sequence
  ABD Primer 21, Synthesized in the Lab
gagaacttgacaaatatggagtaagtgactattacaagaacctaatcaac

SEQ ID NO: 22 - DNA, 50 bp, Artificial Sequence
  ABD Primer 22,  Synthesized in the Lab
tacaccttcaacagttttggcattgttgattaggttcttgtaatagtcac

SEQ ID NO: 23 - DNA, 50 bp, Artificial Sequence
  ABD Primer 23, Synthesized in the Lab
gccaaaactgttgaaggtgtaaaagcactgatagatgaaattttagctgc

SEQ ID NO: 24 - DNA, 50 bp, Artificial Sequence
  ABD Primer 24, Synthesized in the Lab
atggtgatggtgatgatgaggtaatgcagctaaaatttcatctatcagtg

SEQ ID NO: 25 - DNA, 50 bp, Artificial Sequence
  ABD Primer 25, Synthesized in the Lab
catatgttatgcgatggatccagtaacaacaataataacaatggtagcgg

SEQ ID NO: 26 - DNA, 50 bp, Artificial Sequence
  ABD Primer 26, Synthesized in the Lab
tgttcgcatccaccgcttcatcaccgccgctaccattgttattattgttg

SEQ ID NO: 27 - DNA, 50 bp, Artificial Sequence
  ABD Primer 27, Synthesized in the Lab
gaagcggtggatgcgaacagcctggcggaagcgaaagaagcggcgaacgc

SEQ ID NO: 28 - DNA, 50 bp, Artificial Sequence
  ABD Primer 28, Synthesized in the Lab
aaaatcgctcacgccatagctatccagttccgcgttcgccgcttctttcg

SEQ ID NO: 29 - DNA, 50 bp, Artificial Sequence
  ABD Primer 29, Synthesized in the Lab
ctatggcgtgagcgatttttataaacgcctgattgataaagcgaaaaccg

SEQ ID NO: 30 - DNA, 50 bp, Artificial Sequence
  ABD Primer 30, Synthesized in the Lab
tcgcatctttcagcgcttccacgccttccacggttttcgctttatcaatc

SEQ ID NO: 31 - DNA, 50 bp, Artificial Sequence
  ABD Primer 31, Synthesized in the Lab
gaagcgctgaaagatgcgattctggcggcgctgccgcatcatcaccatca

SEQ ID NO: 32 - DNA, 35 bp, Artificial Sequence
  ABD Primer 32, Synthesized in the Lab
ctaaaagcttaatggtgatggtgatgatgcggcag

SEQ ID NO: 33 - DNA, 222 bp, Artificial Sequence
  His-ABD-Linker, Synthesized in the Lab
atgcatcatcaccatcaccatgatgaagccgtggatgcgaattccttagctgaagctaaagtcttagctaacagagaacttgacaaatatggagtaagtgactattacaagaacctaatcaacaatgccaaaactgttgaaggtgtaaaagcactgatagatgaaattttagctgcattaccttcgggtagtaacaacaataataacaatggtagcggcgga

SEQ ID NO: 34 - DNA, 222 bp, Artificial Sequence
  His-ABD094-Linker, Synthesized in the Lab
atgcatcatcaccatcaccatgatgaagcggtggatgcgaacagcctggcggaagcgaaagaagcggcgaacgcggaactggatagctatggcgtgagcgatttttataaacgcctgattgataaagcgaaaaccgtggaaggcgtggaagcgctgaaagatgcgattctggcggcgctgccgtcgggtagtaacaacaataataacaatggtagcggcgga

SEQ ID NO: 35 - DNA, 222 bp, Artificial Sequence
  Linker-ABD-His, Synthesized in the Lab
ggatccagtaacaacaataataacaatggtagcggcggtgatgaagccgtggatgcgaattccttagctgaagctaaagtcttagctaacagagaacttgacaaatatggagtaagtgactattacaagaacctaatcaacaatgccaaaactgttgaaggtgtaaaagcactgatagatgaaattttagctgcattacctcatcatcaccatcaccattaa

SEQ ID NO: 36 - DNA, 222 bp, Artificial Sequence
  Linker-ABD094-His, Synthesized in the Lab
ggatccagtaacaacaataataacaatggtagcggcggtgatgaagcggtggatgcgaacagcctggcggaagcgaaagaagcggcgaacgcggaactggatagctatggcgtgagcgatttttataaacgcctgattgataaagcgaaaaccgtggaaggcgtggaagcgctgaaagatgcgattctggcggcgctgccgcatcatcaccatcaccattaa

SEQ ID NO: 37 - DNA, 1191 bp, Artificial Sequence
  N-ABD-rhArg gene, Synthesized in the Lab
atgcatcatcaccatcaccatgatgaagccgtggatgcgaattccttagctgaagctaaagtcttagctaacagagaacttgacaaatatggagtaagtgactattacaagaacctaatcaacaatgccaaaactgttgaaggtgtaaaagcactgatagatgaaattttagctgcattaccttcgggtagtaacaacaataataacaatggtagcggcggaatgtccgccaagtccagaaccatagggattattggagctcctttctcaaagggacagccacgaggaggggtggaagaaggccctacagtattgagaaaggctggtctgcttgagaaacttaaagaacaagagtgtgatgtgaaggattatggggacctgccctttgctgacatccctaatgacagtccctttcaaattgtgaagaatccaaggtctgtgggaaaagcaagcgagcagctggctggcaaggtggcagaagtcaagaagaacggaagaatcagcctggtgctgggcggagaccacagtttggcaattggaagcatctctggccatgccagggtccaccctgatcttggagtcatctgggtggatgctcacactgatatcaacactccactgacaaccacaagtggaaacttgcatggacaacctgtatctttcctcctgaaggaactaaaaggaaagattcccgatgtgccaggattctcctgggtgactccctgtatatctgccaaggatattgtgtatattggcttgagagacgtggaccctggggaacactacattttgaaaactctaggcattaaatacttttcaatgactgaagtggacagactaggaattggcaaggtgatggaagaaacactcagctatctactaggaagaaagaaaaggccaattcatctaagttttgatgttgacggactggacccatctttcacaccagctactggcacaccagtcgtgggaggtctgacatacagagaaggtctctacatcacagaagaaatctacaaaacagggctactctcaggattagatataatggaagtgaacccatccctggggaagacaccagaagaagtaactcgaacagtgaacacagcagttgcaataaccttggcttgtttcggacttgctcgggagggtaatcacaagcctattgactaccttaacccacctaagtaa

SEQ ID NO: 38 - DNA, 1191 bp, Artificial Sequence
  N-ABD094-rhArg gene, Synthesized in the Lab
atgcatcatcaccatcaccatgatgaagcggtggatgcgaacagcctggcggaagcgaaagaagcggcgaacgcggaactggatagctatggcgtgagcgatttttataaacgcctgattgataaagcgaaaaccgtggaaggcgtggaagcgctgaaagatgcgattctggcggcgctgccgtcgggtagtaacaacaataataacaatggtagcggcggaatgtccgccaagtccagaaccatagggattattggagctcctttctcaaagggacagccacgaggaggggtggaagaaggccctacagtattgagaaaggctggtctgcttgagaaacttaaagaacaagagtgtgatgtgaaggattatggggacctgccctttgctgacatccctaatgacagtccctttcaaattgtgaagaatccaaggtctgtgggaaaagcaagcgagcagctggctggcaaggtggcagaagtcaagaagaacggaagaatcagcctggtgctgggcggagaccacagtttggcaattggaagcatctctggccatgccagggtccaccctgatcttggagtcatctgggtggatgctcacactgatatcaacactccactgacaaccacaagtggaaacttgcatggacaacctgtatctttcctcctgaaggaactaaaaggaaagattcccgatgtgccaggattctcctgggtgactccctgtatatctgccaaggatattgtgtatattggcttgagagacgtggaccctggggaacactacattttgaaaactctaggcattaaatacttttcaatgactgaagtggacagactaggaattggcaaggtgatggaagaaacactcagctatctactaggaagaaagaaaaggccaattcatctaagttttgatgttgacggactggacccatctttcacaccagctactggcacaccagtcgtgggaggtctgacatacagagaaggtctctacatcacagaagaaatctacaaaacagggctactctcaggattagatataatggaagtgaacccatccctggggaagacaccagaagaagtaactcgaacagtgaacacagcagttgcaataaccttggcttgtttcggacttgctcgggagggtaatcacaagcctattgactaccttaacccacctaagtaa

SEQ ID NO: 39 - DNA, 1188 bp, Artificial Sequence
  C-ABD-rhArg gene, Synthesized in the Lab
atgagcgccaagtccagaaccatagggattattggagctcctttctcaaagggacagccacgaggaggggtggaagaaggccctacagtattgagaaaggctggtctgcttgagaaacttaaagaacaagagtgtgatgtgaaggattatggggacctgccctttgctgacatccctaatgacagtccctttcaaattgtgaagaatccaaggtctgtgggaaaagcaagcgagcagctggctggcaaggtggcagaagtcaagaagaacggaagaatcagcctggtgctgggcggagaccacagtttggcaattggaagcatctctggccatgccagggtccaccctgatcttggagtcatctgggtggatgctcacactgatatcaacactccactgacaaccacaagtggaaacttgcatggacaacctgtatctttcctcctgaaggaactaaaaggaaagattcccgatgtgccaggattctcctgggtgactccctgtatatctgccaaggatattgtgtatattggcttgagagacgtggaccctggggaacactacattttgaaaactctaggcattaaatacttttcaatgactgaagtggacagactaggaattggcaaggtgatggaagaaacactcagctatctactaggaagaaagaaaaggccaattcatctaagttttgatgttgacggactggacccatctttcacaccagctactggcacaccagtcgtgggaggtctgacatacagagaaggtctctacatcacagaagaaatctacaaaacagggctactctcaggattagatataatggaagtgaacccatccctggggaagacaccagaagaagtaactcgaacagtgaacacagcagttgcaataaccttggcttgtttcggacttgctcgggagggtaatcacaagcctattgactaccttaacccacctaagggatccagtaacaacaataataacaatggtagcggcggtgatgaagccgtggatgcgaattccttagctgaagctaaagtcttagctaacagagaacttgacaaatatggagtaagtgactattacaagaacctaatcaacaatgccaaaactgttgaaggtgtaaaagcactgatagatgaaattttagctgcattacctcatcatcaccatcaccattaa

SEQ ID NO: 40 - DNA, 1188 bp, Artificial Sequence
  C-ABD094-rhArg gene, Synthesized in the Lab
atgagcgccaagtccagaaccatagggattattggagctcctttctcaaagggacagccacgaggaggggtggaagaaggccctacagtattgagaaaggctggtctgcttgagaaacttaaagaacaagagtgtgatgtgaaggattatggggacctgccctttgctgacatccctaatgacagtccctttcaaattgtgaagaatccaaggtctgtgggaaaagcaagcgagcagctggctggcaaggtggcagaagtcaagaagaacggaagaatcagcctggtgctgggcggagaccacagtttggcaattggaagcatctctggccatgccagggtccaccctgatcttggagtcatctgggtggatgctcacactgatatcaacactccactgacaaccacaagtggaaacttgcatggacaacctgtatctttcctcctgaaggaactaaaaggaaagattcccgatgtgccaggattctcctgggtgactccctgtatatctgccaaggatattgtgtatattggcttgagagacgtggaccctggggaacactacattttgaaaactctaggcattaaatacttttcaatgactgaagtggacagactaggaattggcaaggtgatggaagaaacactcagctatctactaggaagaaagaaaaggccaattcatctaagttttgatgttgacggactggacccatctttcacaccagctactggcacaccagtcgtgggaggtctgacatacagagaaggtctctacatcacagaagaaatctacaaaacagggctactctcaggattagatataatggaagtgaacccatccctggggaagacaccagaagaagtaactcgaacagtgaacacagcagttgcaataaccttggcttgtttcggacttgctcgggagggtaatcacaagcctattgactaccttaacccacctaagggatccagtaacaacaataataacaatggtagcggcggtgatgaagcggtggatgcgaacagcctggcggaagcgaaagaagcggcgaacgcggaactggatagctatggcgtgagcgatttttataaacgcctgattgataaagcgaaaaccgtggaaggcgtggaagcgctgaaagatgcgattctggcggcgctgccgcatcatcaccatcaccattaa

SEQ ID NO: 41 - DNA, 1125 bp, Artificial Sequence
  N-ABD-BCA gene, Synthesized in the Lab
atgcatcatcaccatcaccatgatgaagccgtggatgcgaattccttagctgaagctaaagtcttagctaacagagaacttgacaaatatggagtaagtgactattacaagaacctaatcaacaatgccaaaactgttgaaggtgtaaaagcactgatagatgaaattttagctgcattaccttcgggtagtaacaacaataataacaatggtagcggcggatccatgaagccaatttcaattatcggggttccgatggatttagggcagacacgccgcggcgttgatatggggccgagcgcaatgcgttatgcaggcgtcatcgaacgtctggaacgtcttcattacgatattgaagatttgggagatattccgattggaaaagcagagcggttgcacgagcaaggagattcacggttgcgcaatttgaaagcggttgcggaagcgaacgagaaacttgcggcggcggttgaccaagtcgttcagcgggggcgatttccgcttgtgttgggcggcgaccatagcatcgccattggcacgctcgccggggtggcgaaacattatgagcggcttggagtgatctggtatgacgcgcatggcgacgtcaacaccgcggaaacgtcgccgtctggaaacattcatggcatgccgctggcggcgagcctcgggtttggccatccggcgctgacgcaaatcggcggatacagccccaaaatcaagccggaacatgtcgtgttgatcggcgtccgttcccttgatgaaggggagaagaagtttattcgcgaaaaaggaatcaaaatttacacgatgcatgaggttgatcggctcggaatgacaagggtgatggaagaaacgatcgcctatttaaaagaacgaacggatggcgttcatttgtcgcttgacttggatggccttgacccaagcgacgcaccgggagtcggaacgcctgtcattggaggattgacataccgcgaaagccatttggcgatggagatgctggccgaggcacaaatcatcacttcagcggaatttgtcgaagtgaacccgatcttggatgagcggaacaaaacagcatcagtggctgtagcgctgatggggtcgttgtttggtgaaaaactcatgtaa

SEQ ID NO: 42 - DNA, 1125 bp, Artificial Sequence
  N-ABD094-BCA gene, Synthesized in the Lab
atgcatcatcaccatcaccatgatgaagcggtggatgcgaacagcctggcggaagcgaaagaagcggcgaacgcggaactggatagctatggcgtgagcgatttttataaacgcctgattgataaagcgaaaaccgtggaaggcgtggaagcgctgaaagatgcgattctggcggcgctgccgtcgggtagtaacaacaataataacaatggtagcggcggatccatgaagccaatttcaattatcggggttccgatggatttagggcagacacgccgcggcgttgatatggggccgagcgcaatgcgttatgcaggcgtcatcgaacgtctggaacgtcttcattacgatattgaagatttgggagatattccgattggaaaagcagagcggttgcacgagcaaggagattcacggttgcgcaatttgaaagcggttgcggaagcgaacgagaaacttgcggcggcggttgaccaagtcgttcagcgggggcgatttccgcttgtgttgggcggcgaccatagcatcgccattggcacgctcgccggggtggcgaaacattatgagcggcttggagtgatctggtatgacgcgcatggcgacgtcaacaccgcggaaacgtcgccgtctggaaacattcatggcatgccgctggcggcgagcctcgggtttggccatccggcgctgacgcaaatcggcggatacagccccaaaatcaagccggaacatgtcgtgttgatcggcgtccgttcccttgatgaaggggagaagaagtttattcgcgaaaaaggaatcaaaatttacacgatgcatgaggttgatcggctcggaatgacaagggtgatggaagaaacgatcgcctatttaaaagaacgaacggatggcgttcatttgtcgcttgacttggatggccttgacccaagcgacgcaccgggagtcggaacgcctgtcattggaggattgacataccgcgaaagccatttggcgatggagatgctggccgaggcacaaatcatcacttcagcggaatttgtcgaagtgaacccgatcttggatgagcggaacaaaacagcatcagtggctgtagcgctgatggggtcgttgtttggtgaaaaactcatgtaa

SEQ ID NO: 43 - DNA, 1119 bp, Artificial Sequence
  C-ABD-BCA gene, Synthesized in the Lab
atgaagccaatttcaattatcggggttccgatggatttagggcagacacgccgcggcgttgatatggggccgagcgcaatgcgttatgcaggcgtcatcgaacgtctggaacgtcttcattacgatattgaagatttgggagatattccgattggaaaagcagagcggttgcacgagcaaggagattcacggttgcgcaatttgaaagcggttgcggaagcgaacgagaaacttgcggcggcggttgaccaagtcgttcagcgggggcgatttccgcttgtgttgggcggcgaccatagcatcgccattggcacgctcgccggggtggcgaaacattatgagcggcttggagtgatctggtatgacgcgcatggcgacgtcaacaccgcggaaacgtcgccgtctggaaacattcatggcatgccgctggcggcgagcctcgggtttggccatccggcgctgacgcaaatcggcggatacagccccaaaatcaagccggaacatgtcgtgttgatcggcgtccgttcccttgatgaaggggagaagaagtttattcgcgaaaaaggaatcaaaatttacacgatgcatgaggttgatcggctcggaatgacaagggtgatggaagaaacgatcgcctatttaaaagaacgaacggatggcgttcatttgtcgcttgacttggatggccttgacccaagcgacgcaccgggagtcggaacgcctgtcattggaggattgacataccgcgaaagccatttggcgatggagatgctggccgaggcacaaatcatcacttcagcggaatttgtcgaagtgaacccgatcttggatgagcggaacaaaacagcatcagtggctgtagcgctgatggggtcgttgtttggtgaaaaactcatgggatccagtaacaacaataataacaatggtagcggcggtgatgaagccgtggatgcgaattccttagctgaagctaaagtcttagctaacagagaacttgacaaatatggagtaagtgactattacaagaacctaatcaacaatgccaaaactgttgaaggtgtaaaagcactgatagatgaaattttagctgcattacctcatcatcaccatcaccattaa

SEQ ID NO: 44 - DNA, 1119 bp, Artificial Sequence
  C-ABD094-BCA gene, Synthesized in the Lab
atgaagccaatttcaattatcggggttccgatggatttagggcagacacgccgcggcgttgatatggggccgagcgcaatgcgttatgcaggcgtcatcgaacgtctggaacgtcttcattacgatattgaagatttgggagatattccgattggaaaagcagagcggttgcacgagcaaggagattcacggttgcgcaatttgaaagcggttgcggaagcgaacgagaaacttgcggcggcggttgaccaagtcgttcagcgggggcgatttccgcttgtgttgggcggcgaccatagcatcgccattggcacgctcgccggggtggcgaaacattatgagcggcttggagtgatctggtatgacgcgcatggcgacgtcaacaccgcggaaacgtcgccgtctggaaacattcatggcatgccgctggcggcgagcctcgggtttggccatccggcgctgacgcaaatcggcggatacagccccaaaatcaagccggaacatgtcgtgttgatcggcgtccgttcccttgatgaaggggagaagaagtttattcgcgaaaaaggaatcaaaatttacacgatgcatgaggttgatcggctcggaatgacaagggtgatggaagaaacgatcgcctatttaaaagaacgaacggatggcgttcatttgtcgcttgacttggatggccttgacccaagcgacgcaccgggagtcggaacgcctgtcattggaggattgacataccgcgaaagccatttggcgatggagatgctggccgaggcacaaatcatcacttcagcggaatttgtcgaagtgaacccgatcttggatgagcggaacaaaacagcatcagtggctgtagcgctgatggggtcgttgtttggtgaaaaactcatgggatccagtaacaacaataataacaatggtagcggcggtgatgaagcggtggatgcgaacagcctggcggaagcgaaagaagcggcgaacgcggaactggatagctatggcgtgagcgatttttataaacgcctgattgataaagcgaaaaccgtggaaggcgtggaagcgctgaaagatgcgattctggcggcgctgccgcatcatcaccatcaccattaa

SEQ ID NO: 45 - protein, 74 aa, Artificial Sequence
  His-ABD-Linker, Synthesized in the Lab
MHHHHHHDEAVDANSLAEAKVLANRELDKYGVSDYYKNLINNAKTVEGVKALIDEILAALPSGSNNNNNNGSGG

SEQ ID NO: 46 - protein, 74 aa, Artificial Sequence
  His-ABD094-Linker, Synthesized in the Lab
MHHHHHHDEAVDANSLAEAKEAANAELDSYGVSDFYKRLIDKAKTVEGVEALKDAILAALPSGSNNNNNNGSGG

SEQ ID NO: 47 - protein, 73 aa, Artificial Sequence
  Linker-ABD-His, Synthesized in the Lab
GSSNNNNNNGSGGDEAVDANSLAEAKVLANRELDKYGVSDYYKNLINNAKTVEGVKALIDEILAALPHHHHHH

SEQ ID NO: 48 - protein, 73 aa, Artificial Sequence
  Linker-ABD094-His, Synthesized in the Lab
GSSNNNNNNGSGGDEAVDANSLAEAKEAANAELDSYGVSDFYKRLIDKAKTVEGVEALKDAILAALPHHHHHH

SEQ ID NO: 49 - protein, 396 aa, Artificial Sequence
  N-ABD-rhArg, Synthesized in the Lab
MHHHHHHDEAVDANSLAEAKVLANRELDKYGVSDYYKNLINNAKTVEGVKALIDEILAALPSGSNNNNNNGSGGMSAKSRTIGIIGAPFSKGQPRGGVEEGPTVLRKAGLLEKLKEQECDVKDYGDLPFADIPNDSPFQIVKNPRSVGKASEQLAGKVAEVKKNGRISLVLGGDHSLAIGSISGHARVHPDLGVIWVDAHTDINTPLTTTSGNLHGQPVSFLLKELKGKIPDVPGFSWVTPCISAKDIVYIGLRDVDPGEHYILKTLGIKYFSMTEVDRLGIGKVMEETLSYLLGRKKRPIHLSFDVDGLDPSFTPATGTPVVGGLTYREGLYITEEIYKTGLLSGLDIMEVNPSLGKTPEEVTRTVNTAVAITLACFGLAREGNHKPIDYLNPPK

SEQ ID NO: 50 - protein, 396 aa, Artificial Sequence
  N-ABD094-rhArg, Synthesized in the Lab
MHHHHHHDEAVDANSLAEAKEAANAELDSYGVSDFYKRLIDKAKTVEGVEALKDAILAALPSGSNNNNNNGSGGMSAKSRTIGIIGAPFSKGQPRGGVEEGPTVLRKAGLLEKLKEQECDVKDYGDLPFADIPNDSPFQIVKNPRSVGKASEQLAGKVAEVKKNGRISLVLGGDHSLAIGSISGHARVHPDLGVIWVDAHTDINTPLTTTSGNLHGQPVSFLLKELKGKIPDVPGFSWVTPCISAKDIVYIGLRDVDPGEHYILKTLGIKYFSMTEVDRLGIGKVMEETLSYLLGRKKRPIHLSFDVDGLDPSFTPATGTPVVGGLTYREGLYITEEIYKTGLLSGLDIMEVNPSLGKTPEEVTRTVNTAVAITLACFGLAREGNHKPIDYLNPPK

SEQ ID NO: 51 - protein, 395 aa, Artificial Sequence
  C-ABD-rhArg, Synthesized in the Lab
MSAKSRTIGIIGAPFSKGQPRGGVEEGPTVLRKAGLLEKLKEQECDVKDYGDLPFADIPNDSPFQIVKNPRSVGKASEQLAGKVAEVKKNGRISLVLGGDHSLAIGSISGHARVHPDLGVIWVDAHTDINTPLTTTSGNLHGQPVSFLLKELKGKIPDVPGFSWVTPCISAKDIVYIGLRDVDPGEHYILKTLGIKYFSMTEVDRLGIGKVMEETLSYLLGRKKRPIHLSFDVDGLDPSFTPATGTPVVGGLTYREGLYITEEIYKTGLLSGLDIMEVNPSLGKTPEEVTRTVNTAVAITLACFGLAREGNHKPIDYLNPPKGSSNNNNNNGSGGDEAVDANSLAEAKVLANRELDKYGVSDYYKNLINNAKTVEGVKALIDEILAALPHHHHHH

SEQ ID NO: 52 - protein, 395 aa, Artificial Sequence
  C-ABD094-rhArg, Synthesized in the Lab
MSAKSRTIGIIGAPFSKGQPRGGVEEGPTVLRKAGLLEKLKEQECDVKDYGDLPFADIPNDSPFQIVKNPRSVGKASEQLAGKVAEVKKNGRISLVLGGDHSLAIGSISGHARVHPDLGVIWVDAHTDINTPLTTTSGNLHGQPVSFLLKELKGKIPDVPGFSWVTPCISAKDIVYIGLRDVDPGEHYILKTLGIKYFSMTEVDRLGIGKVMEETLSYLLGRKKRPIHLSFDVDGLDPSFTPATGTPVVGGLTYREGLYITEEIYKTGLLSGLDIMEVNPSLGKTPEEVTRTVNTAVAITLACFGLAREGNHKPIDYLNPPKGSSNNNNNNGSGGDEAVDANSLAEAKEAANAELDSYGVSDFYKRLIDKAKTVEGVEALKDAILAALPHHHHHH

SEQ ID NO: 53 - protein, 374 aa, Artificial Sequence
  N-ABD-BCA, Synthesized in the Lab
MHHHHHHDEAVDANSLAEAKVLANRELDKYGVSDYYKNLINNAKTVEGVKALIDEILAALPSGSNNNNNNGSGGSMKPISIIGVPMDLGQTRRGVDMGPSAMRYAGVIERLERLHYDIEDLGDIPIGKAERLHEQGDSRLRNLKAVAEANEKLAAAVDQVVQRGRFPLVLGGDHSIAIGTLAGVAKHYERLGVIWYDAHGDVNTAETSPSGNIHGMPLAASLGFGHPALTQIGGYSPKIKPEHVVLIGVRSLDEGEKKFIREKGIKIYTMHEVDRLGMTRVMEETIAYLKERTDGVHLSLDLDGLDPSDAPGVGTPVIGGLTYRESHLAMEMLAEAQIITSAEFVEVNPILDERNKTASVAVALMGSLFGEKLM

SEQ ID NO: 54 - protein, 374 aa, Artificial Sequence
  N-ABD094-BCA, Synthesized in the Lab
MHHHHHHDEAVDANSLAEAKEAANAELDSYGVSDFYKRLIDKAKTVEGVEALKDAILAALPSGSNNNNNNGSGGSMKPISIIGVPMDLGQTRRGVDMGPSAMRYAGVIERLERLHYDIEDLGDIPIGKAERLHEQGDSRLRNLKAVAEANEKLAAAVDQVVQRGRFPLVLGGDHSIAIGTLAGVAKHYERLGVIWYDAHGDVNTAETSPSGNIHGMPLAASLGFGHPALTQIGGYSPKIKPEHVVLIGVRSLDEGEKKFIREKGIKIYTMHEVDRLGMTRVMEETIAYLKERTDGVHLSLDLDGLDPSDAPGVGTPVIGGLTYRESHLAMEMLAEAQIITSAEFVEVNPILDERNKTASVAVALMGSLFGEKLM

SEQ ID NO: 55 - protein, 372 aa, Artificial Sequence
  C-ABD-BCA, Synthesized in the Lab
MKPISIIGVPMDLGQTRRGVDMGPSAMRYAGVIERLERLHYDIEDLGDIPIGKAERLHEQGDSRLRNLKAVAEANEKLAAAVDQVVQRGRFPLVLGGDHSIAIGTLAGVAKHYERLGVIWYDAHGDVNTAETSPSGNIHGMPLAASLGFGHPALTQIGGYSPKIKPEHVVLIGVRSLDEGEKKFIREKGIKIYTMHEVDRLGMTRVMEETIAYLKERTDGVHLSLDLDGLDPSDAPGVGTPVIGGLTYRESHLAMEMLAEAQIITSAEFVEVNPILDERNKTASVAVALMGSLFGEKLMGSSNNNNNNGSGGDEAVDANSLAEAKVLANRELDKYGVSDYYKNLINNAKTVEGVKALIDEILAALPHHHHHH

SEQ ID NO: 56 - protein, 372 aa, Artificial Sequence
  C-ABD094-BCA, Synthesized in the Lab
MKPISIIGVPMDLGQTRRGVDMGPSAMRYAGVIERLERLHYDIEDLGDIPIGKAERLHEQGDSRLRNLKAVAEANEKLAAAVDQVVQRGRFPLVLGGDHSIAIGTLAGVAKHYERLGVIWYDAHGDVNTAETSPSGNIHGMPLAASLGFGHPALTQIGGYSPKIKPEHVVLIGVRSLDEGEKKFIREKGIKIYTMHEVDRLGMTRVMEETIAYLKERTDGVHLSLDLDGLDPSDAPGVGTPVIGGLTYRESHLAMEMLAEAQIITSAEFVEVNPILDERNKTASVAVALMGSLFGEKLMGSSNNNNNNGSGGDEAVDANSLAEAKEAANAELDSYGVSDFYKRLIDKAKTVEGVEALKDAILAALPHHHHHH

SEQ ID NO: 57 - DNA, 50 bp, Artificial Sequence
  ABD094-0F Primer, Synthesized in the Lab
attctggcagcgctgccgtcgggtagtaacaacaataataacaatggtag

SEQ ID NO: 58 - DNA, 50 bp, Artificial Sequence
  ABD094-1F Primer, Synthesized in the Lab
aaccgtggaaggtgtggaagcgctgaaagatgcgattctggcagcgctgc

SEQ ID NO: 59 - DNA, 50 bp, Artificial Sequence
  ABD094-2F Primer, Synthesized in the Lab
gatttttataaacgtctgattgataaagcgaaaaccgtggaaggtgtgga

SEQ ID NO: 60 - DNA, 50 bp, Artificial Sequence
  ABD094-3F Primer, Synthesized in the Lab
ctggatagctatggcgtgagcgatttttataaacgtctgattgataaagc

SEQ ID NO: 61 - DNA, 50 bp, Artificial Sequence
  ABD094-4F Primer, Synthesized in the Lab
gcggaagcgaaagaagcagcaaacgcggaactggatagctatggcgtgag

SEQ ID NO: 62 - DNA, 50 bp, Artificial Sequence
  ABD094-5F Primer, Synthesized in the Lab
accatgatgaagccgtggatgcgaattccctggcggaagcgaaagaagca

SEQ ID NO: 63 - DNA, 46 bp, Artificial Sequence
  abdNde-F Primer, Synthesized in the Lab
ggagatatacatatgcatcatcaccatcaccatgatgaagccgtgg

SEQ ID NO: 64 - DNA, 42 bp, Artificial Sequence
  HuArgHinBam-R Primer, Synthesized in the Lab
tgactaccttaacccacctaagtaagcttggatcctgtaacg

SEQ ID NO: 65 - DNA, 1220 bp, Artificial Sequence
  N-ABD094-rhArg gene, Synthesized in the Lab
ggagatatacatatgcatcatcaccatcaccatgatgaagccgtggatgcgaattccctggcggaagcgaaagaagcagcaaacgcggaactggatagctatggcgtgagcgatttttataaacgtctgattgataaagcgaaaaccgtggaaggtgtggaagcgctgaaagatgcgattctggcagcgctgccgtcgggtagtaacaacaataataacaatggtagcggcggtatgagcgccaagtccagaaccatagggattattggagctcctttctcaaagggacagccacgaggaggggtggaagaaggccctacagtattgagaaaggctggtctgcttgagaaacttaaagaacaagagtgtgatgtgaaggattatggggacctgccctttgctgacatccctaatgacagtccctttcaaattgtgaagaatccaaggtctgtgggaaaagcaagcgagcagctggctggcaaggtggcagaagtcaagaagaacggaagaatcagcctggtgctgggcggagaccacagtttggcaattggaagcatctctggccatgccagggtccaccctgatcttggagtcatctgggtggatgctcacactgatatcaacactccactgacaaccacaagtggaaacttgcatggacaacctgtatctttcctcctgaaggaactaaaaggaaagattcccgatgtgccaggattctcctgggtgactccctgtatatctgccaaggatattgtgtatattggcttgagagacgtggaccctggggaacactacattttgaaaactctaggcattaaatacttttcaatgactgaagtggacagactaggaattggcaaggtgatggaagaaacactcagctatctactaggaagaaagaaaaggccaattcatctaagttttgatgttgacggactggacccatctttcacaccagctactggcacaccagtcgtgggaggtctgacatacagagaaggtctctacatcacagaagaaatctacaaaacagggctactctcaggattagatataatggaagtgaacccatccctggggaagacaccagaagaagtaactcgaacagtgaacacagcagttgcaataaccttggcttgtttcggacttgctcgggagggtaatcacaagcctattgactaccttaacccacctaagtaagcttggatcctgtaacg

SEQ ID NO: 66 - protein, 54 aa, Artificial Sequence
  ABD based on Streptococcus sp. G148, Synthesized in the Lab
DEAVDANSLAEAKVLANRELDKYGVSDYYKNLINNAKTVEGVKALIDEILAALP

SEQ ID NO: 67 - protein, 57 aa, Artificial Sequence
  ABD based on Streptococcus sp. G148, Synthesized in the Lab
AQHDEAVDANSLAEAKVLANRELDKYGVSDYYKNLINNAKTVEGVKALIDEILAALP

SEQ ID NO: 68 - protein, 46 aa, Artificial Sequence
  ABD094 Without Linker, Synthesized in Lab
LAEAKEAANAELDSYGVSDFYKRLIDKAKTVEGVEALKDAILAALP

SEQ ID NO: 69 - protein, 324 aa, Homo sapiens
  Xaa (1)..(1): Xaa at position one is either methionine or not present.
XAASAKSRTIGIIGAPFSKGQPRGGVEEGPTVLRKAGLLEKLKEQECDVKDYGDLPFADIPNDSPFQIVKNPRSVGKASEQLAGKVAEVKKNGRISLVLGGDHSLAIGSISGHARVHPDLGVIWVDAHTDINTPLTTTSGNLHGQPVSFLLKELKGKIPDVPGFSWVTPCISAKDIVYIGLRDVDPGEHYILKTLGIKYFSMTEVDRLGIGKVMEETLSYLLGRKKRPIHLSFDVDGLDPSFTPATGTPVVGGLTYREGLYITEEIYKTGLLSGLDIMEVNPSLGKTPEEVTRTVNTAVAITLACFGLAREGNHKPIDYLNPPK

SEQ ID NO: 70 - protein, 299 aa, Bacillus caldovelox
MKPISIIGVPMDLGQTRRGVDMGPSAMRYAGVIERLERLHYDIEDLGDIPIGKAERLHEQGDSRLRNLKAVAEANEKLAAAVDQVVQRGRFPLVLGGDHSIAIGTLAGVAKHYERLGVIWYDAHGDVNTAETSPSGNIHGMPLAASLGFGHPALTQIGGYSPKIKPEHVVLIGVRSLDEGEKKFIREKGIKIYTMHEVDRLGMTRVMEETIAYLKERTDGVHLSLDLDGLDPSDAPGVGTPVIGGLTYRESHLAMEMLAEAQIITSAEFVEVNPILDERNKTASVAVALMGSLFGEKLM

SEQ ID NO: 71 - protein, 299 aa, Artificial Sequence
  BCA (S161C) Arginase, Synthesized in the Lab
MKPISIIGVPMDLGQTRRGVDMGPSAMRYAGVIERLERLHYDIEDLGDIPIGKAERLHEQGDSRLRNLKAVAEANEKLAAAVDQVVQRGRFPLVLGGDHSIAIGTLAGVAKHYERLGVIWYDAHGDVNTAETSPSGNIHGMPLAASLGFGHPALTQIGGYCPKIKPEHVVLIGVRSLDEGEKKFIREKGIKIYTMHEVDRLGMTRVMEETIAYLKERTDGVHLSLDLDGLDPSDAPGVGTPVIGGLTYRESHLAMEMLAEAQIITSAEFVEVNPILDERNKTASVAVALMGSLFGEKLM

SEQ ID NO: 72 - protein, 299 aa, Artificial Sequence
  BCA (V20P, S161C) Arginase, Synthesized in the Lab
MKPISIIGVPMDLGQTRRGPDMGPSAMRYAGVIERLERLHYDIEDLGDIPIGKAERLHEQGDSRLRNLKAVAEANEKLAAAVDQVVQRGRFPLVLGGDHSIAIGTLAGVAKHYERLGVIWYDAHGDVNTAETSPSGNIHGMPLAASLGFGHPALTQIGGYCPKIKPEHVVLIGVRSLDEGEKKFIREKGIKIYTMHEVDRLGMTRVMEETIAYLKERTDGVHLSLDLDGLDPSDAPGVGTPVIGGLTYRESHLAMEMLAEAQIITSAEFVEVNPILDERNKTASVAVALMGSLFGEKLM

SEQ ID NO: 73 - protein, 12 aa, Artificial Sequence
  Linker Sequence 1, Synthesized in the Lab
GSNNNNNNGSGG

SEQ ID NO: 74 - protein, 13 aa, Artificial Sequence
  Linker Sequence 2, Synthesized in the Lab
SGSNNNNNNGSGG

SEQ ID NO: 75 - protein, 362 aa, Artificial Sequence
  BHA Fusion Protein, Synthesized in the Lab
MKPISIIGVPMDLGQTRRGPDMGPSAMRYAGVIERLERLHYDIEDLGDIPIGKAERLHEQGDSRLRNLKAVAEANEKLAAAVDQVVQRGRFPLVLGGDHSIAIGTLAGVAKHYERLGVIWYDAHGDVNTAETSPSGNIHGMPLAASLGFGHPALTQIGGYCPKIKPEHVVLIGVRSLDEGEKKFIREKGIKIYTMHEVDRLGMTRVMEETIAYLKERTDGVHLSLDLDGLDPSDAPGVGTPVIGGLTYRESHLAMEMLAEAQIITSAEFVEVNPILDERNKTASVAVALMGSLFGEKLMHHHHHHAQHDEAVDANSLAEAKVLANRELDKYGVSDYYKNLINNAKTVEGVKALIDEILAALP

SEQ ID NO: 76 - protein, 362 aa, Artificial Sequence
  BAH Fusion Protein, Synthesized in the Lab
MKPISIIGVPMDLGQTRRGPDMGPSAMRYAGVIERLERLHYDIEDLGDIPIGKAERLHEQGDSRLRNLKAVAEANEKLAAAVDQVVQRGRFPLVLGGDHSIAIGTLAGVAKHYERLGVIWYDAHGDVNTAETSPSGNIHGMPLAASLGFGHPALTQIGGYCPKIKPEHVVLIGVRSLDEGEKKFIREKGIKIYTMHEVDRLGMTRVMEETIAYLKERTDGVHLSLDLDGLDPSDAPGVGTPVIGGLTYRESHLAMEMLAEAQIITSAEFVEVNPILDERNKTASVAVALMGSLFGEKLMAQHDEAVDANSLAEAKVLANRELDKYGVSDYYKNLINNAKTVEGVKALIDEILAALPHHHHHH

SEQ ID NO: 77 - DNA, 103 bp, Artificial Sequence
  5'-Sense-ABD Primer, Synthesized in Lab
gcgcagcatgatgaagccgtggatgcgaacagcttagctgaagctaaagtcttagctaacagagaacttgacaaatatggagtaagtgactattacaagaacc

SEQ ID NO: 78 - DNA, 98 bp, Artificial Sequence
  5'-Anti-sense-ABD Primer, Synthesized in the Lab
ttaaggtaatgcagctaaaatttcatctatcagtgcttttacaccttcaacagttttggcattgttgattaggttcttgtaatagtcacttactccat

SEQ ID NO: 79 - DNA, 35 bp, Artificial Sequence
  Forward Primer for Cloning ABD, Synthesized in the Lab
gcatcaccatcaccatcacgcgcagcatgatgaag

SEQ ID NO: 80 - DNA, 38 bp, Artificial Sequence
  Reverse Primer for Cloning ABD, Synthesized in the Lab
cgggatccttaaggtaatgcagctaaaatttcatctat

SEQ ID NO: 81 - DNA, 33 bp, Artificial Sequence
  Forward Primer for Cloning BCA, Synthesized in the Lab
ggaattcccatatgaagccaatttcaattatcg

SEQ ID NO: 82 - DNA, 20 bp, Artificial Sequence
  Reverse Primer for Cloning BCA, Synthesized in the Lab
gtgatggtgatggtgatgca

SEQ ID NO: 83 - DNA, 33 bp, Artificial Sequence; identical to SEQ ID NO: 81
  Forward Primer for Cloning BHA, Synthesized in the Lab

SEQ ID NO: 84 - DNA, 38 bp, Artificial Sequence; identical to SEQ ID NO: 80
  Reverse Primer for Cloning BHA, Synthesized in the Lab

SEQ ID NO: 85 - DNA, 39 bp, Artificial Sequence
  Forward Primer for Cloning ABD, Synthesized in the Lab
cgttgtttggtgaaaaactcatggcgcagcatgatgaag

SEQ ID NO: 86 - DNA, 56 bp, Artificial Sequence
  Reverse Primer for Cloning ABD, Synthesized in the Lab
cgggatccttagtgatggtgatggtgatgaggtaatgcagctaaaatttcatctat

SEQ ID NO: 87 - DNA, 33 bp, Artificial Sequence; identical to SEQ ID NO: 81
  Forward Primer for Cloning BAH, Syntesized in the Lab

SEQ ID NO: 88 - DNA, 56 bp, Artificial Sequence; identical to SEQ ID NO: 86
  Reverse Primer for Cloning BAH, Synthesized in the Lab

SEQ ID NO: 89 - protein, 305 aa, Artificial Sequence
  BCA (S161C) - His, Synthesized in Lab
MKPISIIGVPMDLGQTRRGVDMGPSAMRYAGVIERLERLHYDIEDLGDIPIGKAERLHEQGDSRLRNLKAVAEANEKLAAAVDQVVQRGRFPLVLGGDHSIAIGTLAGVAKHYERLGVIWYDAHGDVNTAETSPSGNIHGMPLAASLGFGHPALTQIGGYCPKIKPEHVVLIGVRSLDEGEKKFIREKGIKIYTMHEVDRLGMTRVMEETIAYLKERTDGVHLSLDLDGLDPSDAPGVGTPVIGGLTYRESHLAMEMLAEAQIITSAEFVEVNPILDERNKTASVAVALMGSLFGEKLMHHHHHH

SEQ ID NO: 90 - DNA, 42 bp, Artificial Sequence
  N-ABDHind-R Primer, Synthesized in the Lab
acagctaaaagcttatcagcctaggatccgccgctaccattg

SEQ ID NO: 91 - DNA, 38 bp, Artificial Sequence
  C-ABDNde-F Primer, Synthesized in the Lab
tagctgatcatatgttatgcgatggatccagtaacaac

SEQ ID NO: 92 - DNA, 33 bp, Artificial Sequence
  C-ABDHind-R, Synthesized in the Lab
gaccctaaaagcttaatggtgatggtgatgatg

SEQ ID NO: 93 - DNA, 34 bp, Artificial Sequence
  HARGBam-F Primer, Synthesized in the Lab
ttagctggggatccgccaagtccagaaccatagg

SEQ ID NO: 94 - DNA, 35 bp, Artificial Sequence
  HARGHind-R Primer, Synthesized in the Lab
gagatcaaagcttacttaggtgggttaaggtagtc

SEQ ID NO: 95 - DNA, 35 bp, Artificial Sequence
  HARGNde-F, Synthesized in the Lab
taggctgcatatgagcgccaagtccagaaccatag

SEQ ID NO: 96 - DNA, 41 bp, Artificial Sequence
  HARGBam-R Primer, Synthesized in the Lab
atcagctaggatcccttaggtgggttaaggtagtcaatagg

SEQ ID NO: 97 - DNA, 36 bp, Artificial Sequence
  BCABam-F Primer, Synthesized in the Lab
atgctagtggatccatgaagccaatttcaattatcg

SEQ ID NO: 98 - DNA, 38 bp, Artificial Sequence
  BCAHind-R Primer, Synthesized in the Lab
tcagcctaaagcttacatgagtttttcaccaaacaacg

SEQ ID NO: 99 - DNA, 35 bp, Artificial Sequence
  BCANde-F Primer, Synthesized in the Lab
atgctagccatatgaagccaatttcaattatcggg

SEQ ID NO: 100 - DNA, 37 bp, Artificial Sequence
  BCABam-R Primer, Synthesized in the Lab
tcagctaaggatcccatgagtttttcaccaaacaacg

SEQ ID NO: 101 - protein, 329 aa, Artificial Sequence
  His-rhArg, Synthesized in Lab
MHHHHHHMSAKSRTIGIIGAPFSKGQPRGGVEEGPTVLRKAGLLEKLKEQECDVKDYGDLPFADIPNDSPFQIVKNPRSVGKASEQLAGKVAEVKKNGRISLVLGGDHSLAIGSISGHARVHPDLGVIWVDAHTDINTPLTTTSGNLHGQPVSFLLKELKGKIPDVPGFSWVTPCISAKDIVYIGLRDVDPGEHYILKTLGIKYFSMTEVDRLGIGKVMEETLSYLLGRKKRPIHLSFDVDGLDPSFTPATGTPVVGGLTYREGLYITEEIYKTGLLSGLDIMEVNPSLGKTPEEVTRTVNTAVAITLACFGLAREGNHKPIDYLNPPK

SEQ ID NO: 102 - protein, 329 aa, Artificial Sequence
  His-rhArg-mono-Cys, Synthesized in Lab
MHHHHHHMSAKSRTIGIIGAPFSKGQPRGGVEEGPTVLRKAGLLEKLKEQECDVKDYGDLPFADIPNDSPFQIVKNPRSVGKASEQLAGKVAEVKKNGRISLVLGGDHSLAIGSISGHARVHPDLGVIWVDAHTDINTPLTTTSGNLHGQPVSFLLKELKGKIPDVPGFSWVTPSISAKDIVYIGLRDVDPGEHYILKTLGIKYFSMTEVDRLGIGKVMEETLSYLLGRKKRPIHLSFDVDGLDPSFTPATGTPVVGGLTYREGLYITEEIYKTGLLSGLDIMEVNPSLGKTPEEVTRTVNTAVAITLASFGLAREGNHKPIDYLNPPK

SEQ ID NO: 103 - protein, 322 aa, Homo sapiens
MSAKSRTIGIIGAPFSKGQPRGGVEEGPTVLRKAGLLEKLKEQECDVKDYGDLPFADIPNDSPFQIVKNPRSVGKASEQLAGKVAEVKKNGRISLVLGGDHSLAIGSISGHARVHPDLGVIWVDAHTDINTPLTTTSGNLHGQPVSFLLKELKGKIPDVPGFSWVTPCISAKDIVYIGLRDVDPGEHYILKTLGIKYFSMTEVDRLGIGKVMEETLSYLLGRKKRPIHLSFDVDGLDPSFTPATGTPVVGGLTYREGLYITEEIYKTGLLSGLDIMEVNPSLGKTPEEVTRTVNTAVAITLACFGLAREGNHKPIDYLNPPK

SEQ ID NO: 104 - protein, 322 aa, Artificial Sequence
  rhArg-mono-Cys, Synthesized in the Lab
MSAKSRTIGIIGAPFSKGQPRGGVEEGPTVLRKAGLLEKLKEQECDVKDYGDLPFADIPNDSPFQIVKNPRSVGKASEQLAGKVAEVKKNGRISLVLGGDHSLAIGSISGHARVHPDLGVIWVDAHTDINTPLTTTSGNLHGQPVSFLLKELKGKIPDVPGFSWVTPSISAKDIVYIGLRDVDPGEHYILKTLGIKYFSMTEVDRLGIGKVMEETLSYLLGRKKRPIHLSFDVDGLDPSFTPATGTPVVGGLTYREGLYITEEIYKTGLLSGLDIMEVNPSLGKTPEEVTRTVNTAVAITLASFGLAREGNHKPIDYLNPPK

SEQ ID NO: 105 - protein, 46 aa, Artificial Sequence
  A(EAAAK)4ALEA-(EAAAK)4A Peptide Linker, Synthesized in the Lab
AEAAAKEAAAKEAAAKEAAAKALEAEAAAKEAAAKEAAAKEAAAKA

SEQ ID NO: 106 - protein, 15 aa, Artificial Sequence
  G4SG4SG3SG Peptide Linker, Synthesized in the Lab
GGGGSGGGGSGGGSG